European Patent Application EP 4 242 225 A1, published September 13, 2023. Title: NANOBODIES AGAINST SEVERE ACCUTE RESPIRATORY SYNDROME CORONAVIRUS 2. Applicant: CONSEJO SUPERIOR DE INVESTIGACIONES CIENTÍFICAS UNIVERSIDAD DE LAS PALMAS DE GRAN CANARIA. Application EP22382222.2. The sequence listing filed with the application follows.

SEQUENCE LISTING (46 sequences)

SEQ ID NO: 1 - protein, 10 aa, Artificial Sequence
  1.10 nanobody CDR1
GYTYSTCRKG

SEQ ID NO: 2 - protein, 9 aa, Artificial Sequence
  1.10 nanobody CDR2
SITADGATY

SEQ ID NO: 3 - protein, 11 aa, Artificial Sequence
  1.10 nanobody CDR3
SVKDFTCTFNS

SEQ ID NO: 4 - protein, 10 aa, Artificial Sequence
  1.26 nanobody CDR1
GYTWSSVCMG

SEQ ID NO: 5 - protein, 10 aa, Artificial Sequence
  1.26 nanobody CDR2
GIPSGRNRPY

SEQ ID NO: 6 - protein, 12 aa, Artificial Sequence
  1.26 nanobody CDR3
PCSAPHDPEYNY

SEQ ID NO: 7 - protein, 10 aa, Artificial Sequence
  1.28 nanobody CDR1
GLTNIRCHMA

SEQ ID NO: 8 - protein, 9 aa, Artificial Sequence
  1.28 nanobody CDR2
RITTNGVTD

SEQ ID NO: 9 - protein, 8 aa, Artificial Sequence
  1.28 nanobody CDR 3
CGFSTTTY

SEQ ID NO: 10 - protein, 10 aa, Artificial Sequence
  1.29 nanobody CDR1
GYTINTDAVA

SEQ ID NO: 11 - protein, 10 aa, Artificial Sequence
  1.29 nanobody CDR 2
VIYTGSGNTN

SEQ ID NO: 12 - protein, 13 aa, Artificial Sequence
  1.29 nanobody CDR 3
SGYYGASGYDFNN

SEQ ID NO: 13 - protein, 11 aa, Artificial Sequence
  2.1 nanobody CDR 1
FGATISSAHMG

SEQ ID NO: 14 - protein, 10 aa, Artificial Sequence
  2.1 nanobody CDR2
FRYTDGSSTY

SEQ ID NO: 15 - protein, 15 aa, Artificial Sequence
  2.1 nanobody CDR 3
SNPSWGRLVGGQYNN

SEQ ID NO: 16 - protein, 11 aa, Artificial Sequence
  2.15 nanobody CDR 1
GYASWARKCIG

SEQ ID NO: 17 - protein, 10 aa, Artificial Sequence
  2.15 nanobody CDR 2
AIFDFDGSTY

SEQ ID NO: 18 - protein, 17 aa, Artificial Sequence
  2.15 nanobody CDR 3
TVAFGTCDNWYRGRGDY

SEQ ID NO: 19 - protein, 10 aa, Artificial Sequence
  2.20 nanobody CDR 1
GYTYNNYYMG

SEQ ID NO: 20 - protein, 9 aa, Artificial Sequence
  2.20 nanobody CDR 2
AINSDGLDT

SEQ ID NO: 21 - protein, 19 aa, Artificial Sequence
  2.20 nanobody CDR 3
TGRTVYYSGYDFRLSVDDY

SEQ ID NO: 22 - protein, 119 aa, Artificial Sequence
  1.10 nanobody variable region
QVQLVESGGGSVQAGGSLRLSCAASGYTYSTCRKGWYRQAPGKERELVASITADGATYYLDSVKGRLTISQDNAKNTVYLQMNSLKPEDTAVYYCAASVKDFTCTFNSWGQGTQVTVSS

SEQ ID NO: 23 - protein, 120 aa, Artificial Sequence
  1.26 nanobody variable region
QVQLVESGGGLVQAGGSLRLSCAATGYTWSSVCMGWFRQAPGKEREGVAGIPSGRNRPYYADSVKGRFTISQDNAKNAVFLLMNSLKPEDTAIYYCAPCSAPHDPEYNYWGQGTQVTVSS

SEQ ID NO: 24 - protein, 116 aa, Artificial Sequence
  1.28 nanobody variable region
QVQLVESGGGSVQAGGSLRLSCAASGLTNIRCHMAWYRQAPGKGRELVSRITTNGVTDYADSVKERFTISRHNAENTVYLQMNSLKPEDTAVYYCAACGFSTTTYWGQGTQVTVSS

SEQ ID NO: 25 - protein, 121 aa, Artificial Sequence
  1.29 nanobody variable region
QVQLVESGGGSVQAGGSLRLSCAASGYTINTDAVAWFRQAPGKGDERVAVIYTGSGNTNYADSVKGRFTISQDNAKNTVYLQMNSLKPEDTALYYCASGYYGASGYDFNNWGQGTQVTVSS

SEQ ID NO: 26 - protein, 123 aa, Artificial Sequence
  2.1 nanobody variable region
QVQLVESGGGSVQAGGSLRLSCAAFGATISSAHMGWFRQAPGKEREGVAFRYTDGSSTYYTTSVRGRFTISQDNAKNTVYLQMNSLKPEDTAMYYCASNPSWGRLVGGQYNNWGQGTQITVSS

SEQ ID NO: 27 - protein, 125 aa, Artificial Sequence
  2.15 nanobody variable region
QVQLVESGGGSVQAGGSLKLSCAASGYASWARKCIGWFRQAPGQEREGVAAIFDFDGSTYYSDSVKGRFTISGDNAKNTVSLQMNSLLPKDTAVYYCTVAFGTCDNWYRGRGDYWGQGTQVTVSS

SEQ ID NO: 28 - protein, 127 aa, Artificial Sequence
  2.20 nanobody variable region
QVQLVESGGGSVQAGGSLRLSCAASGYTYNNYYMGWFRQAPGKEREGVAAINSDGLDTYVADSVKGRFTISRDNAKDTVHLQMNSLKPEDTAIYSCATGRTVYYSGYDFRLSVDDYWGQGTQVTVSS

SEQ ID NO: 29 - protein, 119 aa, Artificial Sequence
  humanized 1.10 nanobody variable region
EVQLVESGGGLVQPGGSLRLSCAASGYTYSTCRKGWYRQAPGKGRELVASITADGATYYLDSVKGRLTISRDNSKNTLYLQMNSLRAEDTAVYYCAASVKDFTCTFNSWGQGTQVTVSS

SEQ ID NO: 30 - protein, 120 aa, Artificial Sequence
  humanized 1.26 nanobody variable region
EVQLVESGGGLVQPGGSLRLSCAATGYTWSSVCMGWFRQAPGKGREGVAGIPSGRNRPYYADSVKGRFTISRDNAKNAVYLQMNSLRAEDTAVYYCAPCSAPHDPEYNYWGQGTQVTVSS

SEQ ID NO: 31 - protein, 121 aa, Artificial Sequence
  Humanized 1.29 nanobody variable region
EVQLVESGGGLVQPGGSLRLSCAASGYTINTDAVAWFRQAPGKGDERVAVIYTGSGNTNYADSVKGRFTISRDNAKNTVYLQMNSLRAEDTAVYYCASGYYGASGYDFNNWGQGTQVTVSS

SEQ ID NO: 32 - protein, 125 aa, Artificial Sequence
  Humanized 2.15 nanobody variable region
EVQLVESGGGLVQPGGSLKLSCAASGYASWARKCIGWFRQAPGQGREGVAAIFDFDGSTYYADSVKGRFTISRDNAKNTLYLQMNSLRAEDTAVYYCTVAFGTCDNWYRGRGDYWGQGTQVTVSS

SEQ ID NO: 33 - protein, 15 aa, Artificial Sequence
  Linker
GGGGSGGGGSGGGGS

SEQ ID NO: 34 - protein, 6 aa, Artificial Sequence
  Thrombin recognition site
LVPRGS

SEQ ID NO: 35 - DNA, 50 bp, Artificial Sequence
  VHHSfi2 primer
gtcctcgcaactgcggcccagccggccatggctcaggtgcagctggtgga

SEQ ID NO: 36 - DNA, 37 bp, Artificial Sequence
  VHHNot2 primer
ggactagtgcggccgctgaggagacggtgacctgggt

SEQ ID NO: 37 - DNA, 39 bp, Artificial Sequence
  Nb1-N2-pIg-AgeI  primer
actgcaaccggtgtacattctcaggtgcagctggtggaa

SEQ ID NO: 38 - DNA, 42 bp, Artificial Sequence
  Nb1-C5-pIg-BamHI primer
actggatccagaaccacttgccgctgaggagacggtgacctg

SEQ ID NO: 39 - DNA, 44 bp, Artificial Sequence
  Nb1-C2-pIg-BamHI primer
tcactcgaggcggatccacgcggaaccagcgctgagacggtgac

SEQ ID NO: 40 - DNA, 75 bp, Artificial Sequence
  BamHI-Nb-N-linker primer
atgggatccggaggtggcgggtccggaggtggcgggtccggaggtggcgggtcccaggtgcagctggtggagtct

SEQ ID NO: 41 - protein, 4 aa, Artificial Sequence
  Furin recognition motif
RRAR

SEQ ID NO: 42 - protein, 4 aa, Artificial Sequence
  GSAS sequence
GSAS

SEQ ID NO: 43 - protein, 9 aa, Artificial Sequence
  HA-tag
YPYDVPDYA

SEQ ID NO: 44 - protein, 125 aa, Artificial Sequence
  1.16 nanobody variable region
QVQLVESGGGSVQAGGSLRLSCAASGNTSKRKCVGWFRRAPGKEREGVTLIYTVGGSTVYADSVKGRFTISQDNAKDTVYLQMNSLKPEDSAMYYCAAESWGRQCNLETHRFTFWGQGTQVTVSS

SEQ ID NO: 45 - protein, 125 aa, Artificial Sequence
  2.11 nanobody variable region
QVQLVESGGGSVQAGGSLRLSCAASGDASNRKCVSWFRRAPGKEREGVALIFPVGSSTAYADSVKGRFTISQDSAKDTVYLQMNNLKPEDSGTYYCAAVSWGGRCNLETQTVTFWGQGTQVTVSS

SEQ ID NO: 46 - protein, 116 aa, Artificial Sequence
  humanVH3
  misc_feature (30)..(34): Xaa can be any naturally occurring amino acid
  misc_feature (49)..(59): Xaa can be any naturally occurring amino acid
  misc_feature (99)..(105): Xaa can be any naturally occurring amino acid
EVQLVESGGGLVQPGGSLRLSCAASFTFSXXXXXWVRQAPGKGLEWVSXXXXXXXXXXXYADSVKGRFTISRDNSKNTLYLQMNSLRAEDTAVYYCARXXXXXXXWGQGTLVTVSS